European Patent Specification EP 3 766 972 B1, published April 23, 2025. Title: Nucleic acid complex. Applicant: National University Corporation Tokyo Medical and Dental University TAKEDA PHARMACEUTICAL COMPANY LIMITED. The sequence listing filed with the application follows.

SEQUENCE LISTING (8 sequences)

SEQ ID NO: 1 - DNA, 16 bp, Artificial
  Synthetic
  misc_feature (2)..(3), (14)..(15): LNA
  misc_feature (1)..(1), (16)..(16): 5-methylcytosine LNA
ctagttcactgaatgc

SEQ ID NO: 2 - RNA, 16 nt, Artificial
  Synthetic
  misc_feature (1)..(3), (14)..(16): 2'-O-Me RNA
gcauucagugaacuag

SEQ ID NO: 3 - DNA, 6982 bp, Mus musculus
  Malat1 non-coding RNA
aggcattcaggcagcgagagcagagcagcgtagagcagcacagctgagctcgtgaggcaggagactcagcccgaggaaatcgcagataagtttttaattaaaaagattgagcagtaaaaagaattagaactctaaacttaagctaatagagtagcttatcgaaatattacttagtcttaataatctaagaagatcttaagagataacatgaaggcttatttaaacagtttgaaaaaggaaatgaggagaaaagtatttgtactgtataatggaggctgaccagagcagtttaggagattgtaaagggaggttttgtgaagttctaaaaggttctagtttgaaggtcggccttgtagattaaaacgaaggttacctaaatagaatctaagtggcatttaaaacagtaaagttgtagagaatagtttgaaaatgaggtgtagttttaaaagattgagaaaagtaggttaagttgacggccgttataaaaatccttcgactggcgcatgtacgtttgaaggcatgagttggaaacagggaagatggaagtgttaggctagccgggcgatggtggcgcacgcctttaatcctagcacttgggaggcagaggcaggcggatttctgagttcgaggccagcctggtctacagagtgagttccaggacagccagggctacacagagaaaccctgtcttgaaaaaacaaaaaggttaggctagtatttggagaaagaagattagaaaatggaagtgaaagacgaagaagacatacaggaaggtgaagaaaaagctgttagagaagataggaaaatagaagacaaagcatctttagaagacagaaaaggtacttaaaggcacaggtagtaggaagccgaagaatagaagatagaaagaagcaagatagaaaaacaaaatggaagttaagacaactttggatgccagcattcaagataggcaaagaagataagattgaggccaaaaggttggataagatataaagtcagaaggaaattatctttaaagccataagttcaaatttctgatggagcgagcagtttagaagagtctttagacagccacatacaagattgaagctagcaatcaaagctactaggactgaagtaaaaagttaaggcagaatgcctttgaagagttagaagaatattaaaagccttaacttgtagcttaattttgcttgatgacaaaaggacttttgataacagtttcaagattgtcagcattttgcattggacttgagctgaggtgcttttaaaatcctaacgactagcattggcagctgacccaggtctacacagaagtgcattcagtgaactaggaagacaggagcggcagacaggagtcccgaagccagtttggtgaagctaggaaggactgaggagccagcagcagcagtgcatggtgaagatagcccaggaaagagtgcggttcggtggaggaagctaggaagaaggagccatacggatgtggtggtgaagctgggaaagggttccaggatggtggagcgagagcgagttggtgatgaagctagctggcggcttggcttgtcaactgcgcggaggaggcgagcaggcattgtggagaggatagatagcggctcctagaccagcatgccagtgtgcaagaaaggctgcagggagagcatgcggtgcggtaacattccttgaggtcggcaacatggtggtggttttctgtaacttggatggtaacttgtttactttgtcttaatagttatgggggagttgtaggcttctgtgtaaagagatatatctggggctgtatgtaggcctttgcgggtgttgtaggtttttctttttcagggttatgtcctcttgcatcttgtcagaagcttttgagggctgactgccaaggcccagaaagaagaatggtagatggcaagttgtctttaaccgctcagaggggaatgaatggtagagccagcacaacctcccagttttgtaagacgttgtagtttgaacagatgacctaccacaagcctcactcctgtgtaggggaggtaattgggcaaagtgcttttgggggaatgggggcaaaatatattttgagttcttttccccttaggtctgtctagaatcctaaaggcagatgactcaagggaaccagaaaaaaggaaatccactctcaggataagcagagctcgccaggtttacagtttgtaggaagtagaggatggatgctagctttcacactgagtgtggaggagctggccatggcggaattgctggtagtttactctttccccctcccttaatgagatttgtaaaatcctaaacacttttacttgaaatatttgggagtggtcttaacagggaggagtgggtgggggaaacgttttttttctaagattttccacagatgctatagttgtgttgacacactgggttagagaaggcgtgtactgctatgctgttggcacgacaccttcagggactggagctgccttttgtccttggaagagttttcccagttgccgctgaagtcagcacagtgcggctttggttcacagtcacctcaggagaacctcaggagcttggctaggccagaggttgaagttaagttttacagcaccgtgatttaaaatatttcattaaaggggaggggtaaaacttagttggctgtggccttgtgtttgggtgggtgggggtgttaggtaattgtttagtttatgatttcagataatcataccagagaacttaaatatttggaaaaacaggaaatctcagctttcaagttggcaagtaactcccaatccagtttttgcttcttttttcctttttctttttttgaggcgggcagctaaggaaggttggttcctctgccggtccctcgaaagcgtagggcttgggggttggtctggtccactgggatgatgtgatgctacagtggggactcttctgaagctgttggatgaatatagattgtagtgtgtggttctcttttgaaatttttttcaggtgacttaatgtatcttaataactactataggaacaaaggaagtggctttaatgaccctgaaggaatttcttctggtgatagcttttatattatcaagtaagagatactatctcagttttgtataagcaagtctttttcctagtgtaggagaaatgattttccttgtgactaaacaagatgtaaaggtatgctttttttcttcttgtgcattgtatacttgtgtttatttgtaacttataatttaagaattatgataattcagcctgaatgtcttttagagggtgggcttttgttgatgagggaggggaaacctttttttttctgtagacctttttcagataacaccatctgagtcataaccagcctggcagtgtgatgacgtagatgcagagggagcagctccttggtgaatgagtgataagtaaaggcagaaaaaataatgtcatgtctccatggggaatgagcatgagccagagattgttcctactgatgaaaagctgcatatgcaaaaatttaagcaaatgaaagcaaccagtataaagttatggcaatacctttaaaagttatggcttatctaccaagctttatccacaaaagtaaagaattgatgaaaaacagtgaagatcaaatgttcatctcaaaactgcttttacaaaagcagaatagaaatgaagtgaaaatgctgcattaagcctggagtaaaaagaagctgagcttgttgagatgagtgggatcgagcggctgcgaggcggtgcagtgtgccaatgtttcgtttgcctcagacaggtttctcttcataagcagaagagttgcttcattccatctcggagcaggaaacagcagactgctgttgacagataagtgtaacttggatctgcagtattgcatgttagggatagataagtgccttttttctctttttccaaaaagacctgtagagctgttgaatgtttgcagctggcccctcttaggcagttcagaattttgagtagttttcccatccagcctcttaaaaattcctaagccttgcaccgatgggctttcatgatgggatagctaataggcttttgcatcgtaaacttcaacacaaaagcctacatgattaatgcctactttaattacattgcttacaagattaaggaatctttatcttgaagaccccatgaaagggatcattatgtgctgaaaattagatgttcatattgctaaaatttaaatgtgctccaatgtacttgtgcttaaaatcattaaattatacaaattaataaaatacttcactagagaatgtatgtatttagaaggctgtctccttatttaaataaagtcttgtttgttgtctgtagttagtgtgggcaattttggggggatgttcttctctaatcttttcagaaacttgacttcgaacacttaagtggaccagatcaggatttgagccagaagaccgaaattaactttaaggcaggaaagacaaattttattctccatgcagtgatgagcatttaataattgcaggcctggcatagaggccgtctaactaaggactaagtaccttaggcaggtgggagatgatggtcagagtaaaaggtaactacatattttgtttccagaaagtcaggggtctaatttgaccatggctaaacatctagggtaagacacttttcccccacatttccaaatatgcatgttgagtttaaatgcttacgatcatctcatccactttagccttttgtcacctcacttgagccacgagtggggtcaggcatgtgggtttaaagagttttcctttgcagagcctcatttcatccttcatggagctgctcaggactttgcatataagcgcttgcctctgtcttctgttctgctagtgagtgtgtgatgtgagaccttgcagtgagtttgtttttcctggaatgtggagggagggggggatggggcttacttgttctagctttttttttacagaccacacagaatgcaggtgtcttgacttcaggtcatgtctgttctttggcaagtaatatgtgcagtactgttccaatctgctgctattagaatgcattgtgacgcgactggagtatgattaaagaaagttgtgtttccccaagtgtttggagtagtggttgttggaggaaaagccatgagtaacaggctgagtgttgaggaaatggctctctgcagctttaagtaacccgtgtttgtgattggagccgagtccctttgctgtgctgccttaggtaaatgtttttgttcatttctggtgaggggggttgggagcactgaagcctttagtctcttccagattcaacttaaaatctgacaagaaataaatcagacaagcaacattcttgaagaaattttaactggcaagtggaaatgttttgaacagttccgtggtctttagtgcattatctttgtgtaggtgttctctctcccctcccttggtcttaattcttacatgcaggaacattgacaacagcagacatctatctattcaaggggccagagaatccagacccagtaaggaaaaatagcccatttactttaaatcgataagtgaagcagacatgccattttcagtgtggggattgggaagccctagttctttcagatgtacttcagactgtagaaggagcttccagttgaattgaaattcaccagtggacaaaatgaggacaacaggtgaacgagccttttcttgtttaagattagctactggtaatctagtgttgaatcctctccagcttcatgctggagcagctagcatgtgatgtaatgttggccttggggtggaggggtgaggtgggcgctaagcctttttttaagatttttcaggtacccctcactaaaggcactgaaggcttaatgtaggacagcggagccttcctgtgtggcaagaatcaagcaagcagtattgtatcgagaccaaagtggtatcatggtcggttttgattagcagtggggactaccctaccgtaacaccttgttggaattgaagcatccaaagaaaatacttgagaggccctgggcttgttttaacatctggaaaaaaggctgtttttatagcagcggttaccagcccaaacctcaagttgtgcttgcaggggagggaaaagggggaaagcgggcaaccagtttccccagcttttccagaatcctgttacaaggtctccccacaagtgatttctctgccacatcgccaccatgggcctttggcctaatcacagacccttcacccctcaccttgatgcagccagtagctggatccttgaggtcacgttgcatatcggtttcaaggtaaccatggtgccaaggtcctgtgggttgcaccagaaaaggccatcaattttccccttgcctgtaatttaacattaaaaccatagctaagatgttttatacatagcacctatgcagagtaaacaaaccagtatgggtatagtatgtttgataccagtgctgggtgggaatgtaggaagtcggatgaaaagcaagcctttgtaggaagttgttggggtgggattgcaaaaattctctgctaagactttttcaggtggacataacagacttggccaagctagcatcttagtggaagcagattcgtcagtagggttgtaaaggtttttcttttcctgagaaaacaaccttttgttttctcaggttttgctttttggcctttccctagctttaaaaaaaaaaaagcaaaagacgctggtggctggcactcctggtttccaggacggggttcaagtccctgcggtgtctttgcttgactcttatatcatgaggccattacatttttcttggagggttctaaaggctctgggtatggtagctgatatcactggaacactccccagcctcagtgttgaactcttgataattaactgcattgtctttcaggttatgcccaattcgtcttattacctctgagtcgacacacctcctactatttattgaatactttgattttatgaaataaaaactaaatatctctca

SEQ ID NO: 4 - DNA, 8758 bp, Homo sapiens
  Malat1 non-coding RNA
gtaaaggactggggccccgcaactggcctctcctgccctcttaagcgcagcgccattttagcaacgcagaagcccggcgccgggaagcctcagctcgcctgaaggcaggtcccctctgacgcctccgggagcccaggtttcccagagtccttgggacgcagcgacgagttgtgctgctatcttagctgtccttataggctggccattccaggtggtggtatttagataaaaccactcaaactctgcagtttggtcttggggtttggaggaaagcttttatttttcttcctgctccggttcagaaggtctgaagctcatacctaaccaggcataacacagaatctgcaaaacaaaaacccctaaaaaagcagacccagagcagtgtaaacacttctgggtgtgtccctgactggctgcccaaggtctctgtgtcttcggagacaaagccattcgcttagttggtctactttaaaaggccacttgaactcgctttccatggcgatttgccttgtgagcactttcaggagagcctggaagctgaaaaacggtagaaaaatttccgtgcgggccgtggggggctggcggcaactggggggccgcagatcagagtgggccactggcagccaacggcccccggggctcaggcggggagcagctctgtggtgtgggattgaggcgttttccaagagtgggttttcacgtttctaagatttcccaagcagacagcccgtgctgctccgatttctcgaacaaaaaagcaaaacgtgtggctgtcttgggagcaagtcgcaggactgcaagcagttgggggagaaagtccgccattttgccacttctcaaccgtccctgcaaggctggggctcagttgcgtaatggaaagtaaagccctgaactatcacactttaatcttccttcaaaaggtggtaaactatacctactgtccctcaagagaacacaagaagtgctttaagaggtattttaaaagttccgggggttttgtgaggtgtttgatgacccgtttaaaatatgatttccatgtttcttttgtctaaagtttgcagctcaaatctttccacacgctagtaatttaagtatttctgcatgtgtagtttgcattcaagttccataagctgttaagaaaaatctagaaaagtaaaactagaacctatttttaaccgaagaactactttttgcctccctcacaaaggcggcggaaggtgatcgaattccggtgatgcgagttgttctccgtctataaatacgcctcgcccgagctgtgcggtaggcattgaggcagccagcgcaggggcttctgctgagggggcaggcggagcttgaggaaaccgcagataagtttttttctctttgaaagatagagattaatacaactacttaaaaaatatagtcaataggttactaagatattgcttagcgttaagtttttaacgtaattttaatagcttaagattttaagagaaaatatgaagacttagaagagtagcatgaggaaggaaaagataaaaggtttctaaaacatgacggaggttgagatgaagcttcttcatggagtaaaaaatgtatttaaaagaaaattgagagaaaggactacagagccccgaattaataccaatagaagggcaatgcttttagattaaaatgaaggtgacttaaacagcttaaagtttagtttaaaagttgtaggtgattaaaataatttgaaggcgatcttttaaaaagagattaaaccgaaggtgattaaaagaccttgaaatccatgacgcagggagaattgcgtcatttaaagcctagttaacgcatttactaaacgcagacgaaaatggaaagattaattgggagtggtaggatgaaacaatttggagaagatagaagtttgaagtggaaaactggaagacagaagtacgggaaggcgaagaaaagaatagagaagatagggaaattagaagataaaaacatacttttagaagaaaaaagataaatttaaacctgaaaagtaggaagcagaagaaaaaagacaagctaggaaacaaaaagctaagggcaaaatgtacaaacttagaagaaaattggaagatagaaacaagatagaaaatgaaaatattgtcaagagtttcagatagaaaatgaaaaacaagctaagacaagtattggagaagtatagaagatagaaaaatataaagccaaaaattggataaaatagcactgaaaaaatgaggaaattattggtaaccaatttattttaaaagcccatcaatttaatttctggtggtgcagaagttagaaggtaaagcttgagaagatgagggtgtttacgtagaccagaaccaatttagaagaatacttgaagctagaaggggaagttggttaaaaatcacatcaaaaagctactaaaaggactggtgtaatttaaaaaaaactaaggcagaaggcttttggaagagttagaagaatttggaaggccttaaatatagtagcttagtttgaaaaatgtgaaggactttcgtaacggaagtaattcaagatcaagagtaattaccaacttaatgtttttgcattggactttgagttaagattattttttaaatcctgaggactagcattaattgacagctgacccaggtgctacacagaagtggattcagtgaatctaggaagacagcagcagacaggattccaggaaccagtgtttgatgaagctaggactgaggagcaagcgagcaagcagcagttcgtggtgaagataggaaaagagtccaggagccagtgcgatttggtgaaggaagctaggaagaaggaaggagcgctaacgatttggtggtgaagctaggaaaaaggattccaggaaggagcgagtgcaatttggtgatgaaggtagcaggcggcttggcttggcaaccacacggaggaggcgagcaggcgttgtgcgtagaggatcctagaccagcatgccagtgtgccaaggccacagggaaagcgagtggttggtaaaaatccgtgaggtcggcaatatgttgtttttctggaacttacttatggtaaccttttatttattttctaatataatgggggagtttcgtactgaggtgtaaagggatttatatggggacgtaggccgatttccgggtgttgtaggtttctctttttcaggcttatactcatgaatcttgtctgaagcttttgagggcagactgccaagtcctggagaaatagtagatggcaagtttgtgggttttttttttttacacgaatttgaggaaaaccaaatgaatttgatagccaaattgagacaatttcagcaaatctgtaagcagtttgtatgtttagttggggtaatgaagtatttcagttttgtgaatagatgacctgtttttacttcctcaccctgaattcgttttgtaaatgtagagtttggatgtgtaactgaggcgggggggagttttcagtatttttttttgtgggggtgggggcaaaatatgttttcagttctttttcccttaggtctgtctagaatcctaaaggcaaatgactcaaggtgtaacagaaaacaagaaaatccaatatcaggataatcagaccaccacaggtttacagtttatagaaactagagcagttctcacgttgaggtctgtggaagagatgtccattggagaaatggctggtagttactcttttttccccccacccccttaatcagactttaaaagtgcttaaccccttaaacttgttattttttacttgaagcattttgggatggtcttaacagggaagagagagggtgggggagaaaatgtttttttctaagattttccacagatgctatagtactattgacaaactgggttagagaaggagtgtaccgctgtgctgttggcacgaacaccttcagggactggagctgcttttatccttggaagagtattcccagttgaagctgaaaagtacagcacagtgcagctttggttcatattcagtcatctcaggagaacttcagaagagcttgagtaggccaaatgttgaagttaagttttccaataatgtgacttcttaaaagttttattaaaggggaggggcaaatattggcaattagttggcagtggcctgttacggttgggattggtggggtgggtttaggtaattgtttagtttatgattgcagataaactcatgccagagaacttaaagtcttagaatggaaaaagtaaagaaatatcaacttccaagttggcaagtaactcccaatgatttagtttttttccccccagtttgaattgggaagctgggggaagttaaatatgagccactgggtgtaccagtgcattaatttgggcaaggaaagtgtcataatttgatactgtatctgttttccttcaaagtatagagcttttggggaaggaaagtattgaactgggggttggtctggcctactgggctgacattaactacaattatgggaaatgcaaaagttgtttggatatggtagtgtgtggttctcttttggaatttttttcaggtgatttaataataatttaaaactactatagaaactgcagagcaaaggaagtggcttaatgatcctgaagggatttcttctgatggtagcttttgtattatcaagtaagattctattttcagttgtgtgtaagcaagtttttttttagtgtaggagaaatacttttccattgtttaactgcaaaacaagatgttaaggtatgcttcaaaaattttgtaaattgtttattttaaacttatctgtttgtaaattgtaactgattaagaattgtgatagttcagcttgaatgtctcttagagggtgggcttttgttgatgagggaggggaaactttttttttttctatagacttttttcagataacatcttctgagtcataaccagcctggcagtatgatggcctagatgcagagaaaacagctccttggtgaattgataagtaaaggcagaaaagattatatgtcatacctccattggggaataagcataaccctgagattcttactactgatgagaacattatctgcatatgccaaaaaattttaagcaaatgaaagctaccaatttaaagttacggaatctaccattttaaagttaattgcttgtcaagctataaccacaaaaataatgaattgatgagaaatacaatgaagaggcaatgtccatctcaaaatactgcttttacaaaagcagaataaaagcgaaaagaaatgaaaatgttacactacattaatcctggaataaaagaagccgaaataaatgagagatgagttgggatcaagtggattgaggaggctgtgctgtgtgccaatgtttcgtttgcctcagacaggtatctcttcgttatcagaagagttgcttcatttcatctgggagcagaaaacagcaggcagctgttaacagataagtttaacttgcatctgcagtattgcatgttagggataagtgcttatttttaagagctgtggagttcttaaatatcaaccatggcactttctcctgaccccttccctaggggatttcaggattgagaaatttttccatcgagcctttttaaaattgtaggacttgttcctgtgggcttcagtgatgggatagtacacttcactcagaggcatttgcatctttaaataatttcttaaaagcctctaaagtgatcagtgccttgatgccaactaaggaaatttgtttagcattgaatctctgaaggctctatgaaaggaatagcatgatgtgctgttagaatcagatgttactgctaaaatttacatgttgtgatgtaaattgtgtagaaaaccattaaatcattcaaaataataaactatttttattagagaatgtatacttttagaaagctgtctccttatttaaataaaatagtgtttgtctgtagttcagtgttggggcaatcttgggggggattcttctctaatctttcagaaactttgtctgcgaacactctttaatggaccagatcaggatttgagcggaagaacgaatgtaactttaaggcaggaaagacaaattttattcttcataaagtgatgagcatataataattccaggcacatggcaatagaggccctctaaataaggaataaataacctcttagacaggtgggagattatgatcagagtaaaaggtaattacacattttatttccagaaagtcaggggtctataaattgacagtgattagagtaatactttttcacatttccaaagtttgcatgttaactttaaatgcttacaatcttagagtggtaggcaatgttttacactattgaccttatatagggaagggagggggtgcctgtggggttttaaagaattttcctttgcagaggcatttcatccttcatgaagccattcaggattttgaattgcatatgagtgcttggctcttccttctgttctagtgagtgtatgagaccttgcagtgagtttatcagcatactcaaaatttttttcctggaatttggagggatgggaggagggggtggggcttacttgttgtagctttttttttttttacagacttcacagagaatgcagttgtcttgacttcaggtctgtctgttctgttggcaagtaaatgcagtactgttctgatcccgctgctattagaatgcattgtgaaacgactggagtatgattaaaagttgtgttccccaatgcttggagtagtgattgttgaaggaaaaaatccagctgagtgataaaggctgagtgttgaggaaatttctgcagttttaagcagtcgtatttgtgattgaagctgagtacattttgctggtgtatttttaggtaaaatgctttttgttcatttctggtggtgggaggggactgaagcctttagtcttttccagatgcaaccttaaaatcagtgacaagaaacattccaaacaagcaacagtcttcaagaaattaaactggcaagtggaaatgtttaaacagttcagtgatctttagtgcattgtttatgtgtgggtttctctctcccctcccttggtcttaattcttacatgcaggaacactcagcagacacacgtatgcgaagggccagagaagccagacccagtaagaaaaaatagcctatttactttaaataaaccaaacattccattttaaatgtggggattgggaaccactagttctttcagatggtattcttcagactatagaaggagcttccagttgaattcaccagtggacaaaatgaggaaaacaggtgaacaagctttttctgtatttacatacaaagtcagatcagttatgggacaatagtattgaatagatttcagctttatgctggagtaactggcatgtgagcaaactgtgttggcgtgggggtggaggggtgaggtgggcgctaagcctttttttaagatttttcaggtacccctcactaaaggcaccgaaggcttaaagtaggacaaccatggagccttcctgtggcaggagagacaacaaagcgctattatcctaaggtcaagagaagtgtcagcctcacctgatttttattagtaatgaggacttgcctcaactccctctttctggagtgaagcatccgaaggaatgcttgaagtacccctgggcttctcttaacatttaagcaagctgtttttatagcagctcttaataataaagcccaaatctcaagcggtgcttgaaggggagggaaagggggaaagcgggcaaccacttttccctagcttttccagaagcctgttaaaagcaaggtctccccacaagcaacttctctgccacatcgccaccccgtgccttttgatctagcacagacccttcacccctcacctcgatgcagccagtagcttggatccttgtgggcatgatccataatcggtttcaaggtaacgatggtgtcgaggtctttggtgggttgaactatgttagaaaaggccattaatttgcctgcaaattgttaacagaagggtattaaaaccacagctaagtagctctattataatacttatccagtgactaaaaccaacttaaaccagtaagtggagaaataacatgttcaagaactgtaatgctgggtgggaacatgtaacttgtagactggagaagataggcatttgagtggctgagagggcttttgggtgggaatgcaaaaattctctgctaagactttttcaggtgaacataacagacttggccaagctagcatcttagcggaagctgatctccaatgctcttcagtagggtcatgaaggtttttcttttcctgagaaaacaacacgtattgttttctcaggttttgctttttggcctttttctagcttaaaaaaaaaaaaagcaaaagatgctggtggttggcactcctggtttccaggacggggttcaaatccctgcggcgtctttgctttgactactaatctgtcttcaggactctttctgtatttctccttttctctgcaggtgctagttcttggagttttggggaggtgggaggtaacagcacaatatctttgaactatatacatccttgatgtataatttgtcaggagcttgacttgattgtatattcatatttacacgagaacctaatataactgccttgtctttttcaggtaatagcctgcagctggtgttttgagaagccctactgctgaaaacttaacaattttgtgtaataaaaatggagaagctctaaattgttgtggttcttttgtgaataaaaaaatcttgattggggaaaaaaaaa

SEQ ID NO: 5 - DNA, 2534 bp, Mus musculus
  SR-B1 mRNA
ggaatcccgcgccgaactcgggggcgggctgcccgggccatggcgcataaagcctctggccacctgcagggctactgctgctccggccaccgccaggcacacaccttgctgctgagggagtctcggcttctgtcatctctgtggcctccgtcacctctgtctccgtctccttcaggtcctgagccccgagagccccttccgcgcacgcggacatgggcggcagctccagggcgcgctgggtggccttggggttgggcgccctggggctgctgtttgctgcgctcggcgttgtcatgatcctcatggtgccctccctcatcaagcagcaggtgctcaagaatgtccgcatagacccgagcagcctgtccttcgggatgtggaaggagatccccgtccctttctacttgtctgtctacttcttcgaagtggtcaacccaaacgaggtcctcaacggccagaagccagtagtccgggagcgtggaccctatgtctacagggagttcagacaaaaggtcaacatcaccttcaatgacaacgacaccgtgtccttcgtggagaaccgcagcctccatttccagcctgacaagtcgcatggctcagagagtgactacattgtactgcctaacatcttggtcctggggggctcgatattgatggagagcaagcctgtgagcctgaagctgatgatgaccttggcgctggtcaccatgggccagcgtgcttttatgaaccgcacagttggtgagatcctgtggggctatgacgatcccttcgtgcattttctcaacacgtacctcccagacatgcttcccataaagggcaaatttggcctgtttgttgggatgaacaactcgaattctggggtcttcactgtcttcacgggcgtccagaatttcagcaggatccatctggtggacaaatggaacggactcagcaagatcgattattggcattcagagcagtgtaacatgatcaatgggacttccgggcagatgtgggcacccttcatgacacccgaatcctcgctggaattcttcagcccggaggcatgcaggtccatgaagctgacctacaacgaatcaagggtgtttgaaggcattcccacgtatcgcttcacggcccccgatactctgtttgccaacgggtccgtctacccacccaacgaaggcttctgcccatgccgagagtctggcattcagaatgtcagcacctgcaggtttggtgcgcctctgtttctctcccacccccacttttacaacgccgaccctgtgttgtcagaagctgttcttggtctgaaccctaacccaaaggagcattccttgttcctagacatccatccggtcactgggatccccatgaactgttctgtgaagatgcagctgagcctctacatcaaatctgtcaagggcatcgggcaaacagggaagatcgagccagtagttctgccgttgctgtggttcgaacagagcggagcaatgggtggcaagcccctgagcacgttctacacgcagctggtgctgatgccccaggttcttcactacgcgcagtatgtgctgctggggcttggaggcctcctgttgctggtgcccatcatctgccaactgcgcagccaggagaaatgctttttgttttggagtggtagtaaaaagggctcccaggataaggaggccattcaggcctactctgagtccctgatgtcaccagctgccaagggcacggtgctgcaagaagccaagctatagggtcctgaagacactataagccccccaaacctgatagcttggtcagaccagccacccagtccctacaccccgcttcttgaggactctctcagcggacagcccaccagtgccatggcctgagcccccagatgtcacacctgtccgcacgcacggcacatggatgcccacgcatgtgcaaaaacaactcagggaccagggacagacctgctgccaagtgagcctgatgggccacaggtgtgctcttctaaatggcctgtgagccaggctgtgggaactctagctgctgtcagcccctcctgtaggagctggccctgcccaggctcctgacttccctcaggaagtctttctgtctttctccatcagtctgaaagccttagttcccacagaggacggatctgtcactcctaggggctgggcatatgtcggcctcttgtgccaaggccaggcaagcagctccaggtcctgaccagtttgcacacacactctggagctgtatctggcgctttttctatcgtctctgctatgtcactgaattaaccactgtacgtggcagaggtggcaggcccctcagggtccttatttttcaggcatggggtcaaagctagaggtatgggccgtctacacccccccgccccccggcatctagtgtacctcaccagagggtattcggaggcccagcatcctgcaaccgaccccttttttctactggaagagaaattttatcatcttttgaaaggaagtcatgactgaagcaataaaccttttcactgattcaacaaaaaaaaaaaaaaa

SEQ ID NO: 6 - DNA, 2759 bp, Homo sapiens
  SR-B1 mRNA
gctcaggccccgcccctgccgccggaatcctgaagcccaaggctgcccgggggcggtccggcggcgccggcgatggggcataaaaccactggccacctgccgggctgctcctgcgtgcgctgccgtcccggatccaccgtgcctctgcggcctgcgtgcccggagtccccgcctgtgtcgtctctgtcgccgtccccgtctcctgccaggcgcggagccctgcgagccgcgggtgggccccaggcgcgcagacatgggctgctccgccaaagcgcgctgggctgccggggcgctgggcgtcgcggggctactgtgcgctgtgctgggcgctgtcatgatcgtgatggtgccgtcgctcatcaagcagcaggtccttaagaacgtgcgcatcgaccccagtagcctgtccttcaacatgtggaaggagatccctatccccttctatctctccgtctacttctttgacgtcatgaaccccagcgagatcctgaagggcgagaagccgcaggtgcgggagcgcgggccctacgtgtacagggagttcaggcacaaaagcaacatcaccttcaacaacaacgacaccgtgtccttcctcgagtaccgcaccttccagttccagccctccaagtcccacggctcggagagcgactacatcgtcatgcccaacatcctggtcttgggtgcggcggtgatgatggagaataagcccatgaccctgaagctcatcatgaccttggcattcaccaccctcggcgaacgtgccttcatgaaccgcactgtgggtgagatcatgtggggctacaaggacccccttgtgaatctcatcaacaagtactttccaggcatgttccccttcaaggacaagttcggattatttgctgagctcaacaactccgactctgggctcttcacggtgttcacgggggtccagaacatcagcaggatccacctcgtggacaagtggaacgggctgagcaaggttgacttctggcattccgatcagtgcaacatgatcaatggaacttctgggcaaatgtggccgcccttcatgactcctgagtcctcgctggagttctacagcccggaggcctgccgatccatgaagctaatgtacaaggagtcaggggtgtttgaaggcatccccacctatcgcttcgtggctcccaaaaccctgtttgccaacgggtccatctacccacccaacgaaggcttctgcccgtgcctggagtctggaattcagaacgtcagcacctgcaggttcagtgcccccttgtttctctcccatcctcacttcctcaacgctgacccggttctggcagaagcggtgactggcctgcaccctaaccaggaggcacactccttgttcctggacatccacccggtcacgggaatccccatgaactgctctgtgaaactgcagctgagcctctacatgaaatctgtcgcaggcattggacaaactgggaagattgagcctgtggtcctgccgctgctctggtttgcagagagcggggccatggagggggagactcttcacacattctacactcagctggtgttgatgcccaaggtgatgcactatgcccagtacgtcctcctggcgctgggctgcgtcctgctgctggtccctgtcatctgccaaatccggagccaagagaaatgctatttattttggagtagtagtaaaaagggctcaaaggataaggaggccattcaggcctattctgaatccctgatgacatcagctcccaagggctctgtgctgcaggaagcaaaactgtagggtcctgaggacaccgtgagccagccaggcctggccgctgggcctgaccggccccccagcccctacaccccgcttctcccggactctcccagcggacagccccccagccccacagcctgagcctcccagctgccatgtgcctgttgcacacctgcacacacgccctggcacacatacacacatgcgtgcaggcttgtgcagacactcagggatggagctgctgctgaagggacttgtagggagaggctcgtcaacaagcactgttctggaaccttctctccacgtggcccacaggcctgaccacaggggctgtgggtcctgcgtccccttcctcgggtgagcctggcctgtcccgttcagccgttgggcccaggcttcctcccctccaaggtgaaacactgcagtcccggtgtggtggctccccatgcaggacgggccaggctgggagtgccgccttcctgtgccaaattcagtggggactcagtgcccaggccctggccacgagctttggccttggtctacctgccaggccaggcaaagcgcctttacacaggcctcggaaaacaatggagtgagcacaagatgccctgtgcagctgcccgagggtctccgcccaccccggccggactttgatccccccgaagtcttcacaggcactgcatcgggttgtctggcgcccttttcctccagcctaaactgacatcatcctatggactgagccggccactctctggccgaagtggccgcaggctgtgcccccgagctgcccccaccccctcacagggtccctcagattataggtgcccaggctgaggtgaagaggcctgggggccctgccttccgggcgctcctggaccctggggcaaacctgtgacccttttctactggaatagaaatgagttttatcatctttgaaaaataattcactcttgaagtaataaacgtttaaaaaaatgggaaaaaaaaaaaaaaaaaa

SEQ ID NO: 7 - DNA, 2761 bp, Mus musculus
  DMPK mRNA
gaactggccagagagacccaagggatagtcagggacgggcagacatgcagctagggttctggggcctggacaggggcagccaggccctgtgacgggaagaccccgagctccggcccggggaggggccatggtgttgcctgcccaacatgtcagccgaagtgcggctgaggcagctccagcagctggtgctggacccaggcttcctgggactggagcccctgctcgaccttctcctgggcgtccaccaggagctgggtgcctctcacctagcccaggacaagtatgtggccgacttcttgcagtgggtggagcccattgcagcaaggcttaaggaggtccgactgcagagggatgattttgagattttgaaggtgatcgggcgtggggcgttcagcgaggtagcggtggtgaagatgaaacagacgggccaagtgtatgccatgaagattatgaataagtgggacatgctgaagagaggcgaggtgtcgtgcttccgggaagaaagggatgtattagtgaaaggggaccggcgctggatcacacagctgcactttgccttccaggatgagaactacctgtacctggtcatggaatactacgtgggcggggacctgctaacgctgctgagcaagtttggggagcggatccccgccgagatggctcgcttctacctggccgagattgtcatggccatagactccgtgcaccggctgggctacgtgcacagggacatcaaaccagataacattctgctggaccgatgtgggcacattcgcctggcagacttcggctcctgcctcaaactgcagcctgatggaatggtgaggtcgctggtggctgtgggcaccccggactacctgtctcctgagattctgcaggccgttggtggagggcctggggcaggcagctacgggccagagtgtgactggtgggcactgggcgtgttcgcctatgagatgttctatgggcagacccccttctacgcggactccacagccgagacatatgccaagattgtgcactacagggaacacttgtcgctgccgctggcagacacagttgtccccgaggaagctcaggacctcattcgtgggctgctgtgtcctgctgagataaggctaggtcgaggtggggcaggtgatttccagaaacatcctttcttctttggccttgattgggagggtctccgagacagtgtacccccctttacaccagacttcgagggtgccacggacacatgcaatttcgatgtggtggaggaccggctcactgccatggtgagcgggggcggggagacgctgtcagacatgcaggaagacatgccccttggggtgcgcctgcccttcgtgggctactcctactgctgcatggccttcagagacaatcaggtcccggaccccacccctatggaactagaggccctgcagttgcctgtgtcagacttgcaagggcttgacttgcagcccccagtgtccccaccggatcaagtggctgaagaggctgacctagtggctgtccctgcccctgtggctgaggcagagaccacggtaacgctgcagcagctccaggaagccctggaagaagaggttctcacccggcagagcctgagccgcgagctggaggccatccggaccgccaaccagaacttctccagccaactacaggaggccgaggtccgaaaccgagacctggaggcgcatgttcggcagctacaggaacggatggagatgctgcaggccccaggagccgcagccatcacgggggtccccagtccccgggccacggatccaccttcccatctagatggccccccggccgtggctgtgggccagtgcccgctggtggggccaggccccatgcaccgccgtcacctgctgctccctgccaggatccctaggcctggcctatccgaggcgcgttgcctgctcctgttcgccgctgctctggctgctgccgccacactgggctgcactgggttggtggcctataccggcggtctcaccccagtctggtgtttcccgggagccaccttcgccccctgaaccctaagactccaagccatctttcatttaggcctcctaggaaggtcgagcgaccagggagcgacccaaagcgtctctgtgcccatcgcgccccccccccccccccaccgctccgctccacacttctgtgagcctgggtccccacccagctccgctcctgtgatccaggcctgccacctggcggccggggagggaggaacagggctcgtgcccagcacccctggttcctgcagagctggtagccaccgctgctgcagcagctgggcattcgccgaccttgctttactcagccccgacgtggatgggcaaactgctcagctcatccgatttcactttttcactctcccagccatcagttacaagccataagcatgagccccctatttccagggacatcccattcccatagtgatggatcagcaagacctctgccagcacacacggagtctttggcttcggacagcctcactcctgggggttgctgcaactccttccccgtgtacacgtctgcactctaacaacggagccacagctgcactcccccctcccccaaagcagtgtgggtatttattgatcttgttatctgactcactgacagactccgggacccacgttttagatgcattgagactcgacattcctcggtatttattgtctgtccccacctacgacctccactcccgacccttgcgaataaaatacttctggtctgccctaaa

SEQ ID NO: 8 - DNA, 3243 bp, Homo sapiens
  DMPK mRNA
gccacaagcctccaccccagctggtcccccacccaggctgcccagtttaacattcctagtcataggaccttgacttctgagaggcctgattgtcatctgtaaataaggggtaggactaaagcactcctcctggaggactgagagatgggctggaccggagcacttgagtctgggatatgtgaccatgctacctttgtctccctgtcctgttccttcccccagccccaaatccagggttttccaaagtgtggttcaagaaccacctgcatctgaatctagaggtactggatacaaccccacgtctgggccgttacccaggacattctacatgagaacgtgggggtggggccctggctgcacctgaactgtcacctggagtcagggtggaaggtggaagaactgggtcttatttccttctccccttgttctttagggtctgtccttctgcagactccgttaccccaccctaaccatcctgcacacccttggagccctctgggccaatgccctgtcccgcaaagggcttctcaggcatctcacctctatgggagggcatttttggcccccagaaccttacacggtgtttatgtggggaagcccctgggaagcagacagtcctagggtgaagctgagaggcagagagaaggggagacagacagagggtggggctttcccccttgtctccagtgccctttctggtgaccctcggttcttttcccccaccacccccccagcggagcccatcgtggtgaggcttaaggaggtccgactgcagagggacgacttcgagattctgaaggtgatcggacgcggggcgttcagcgaggtagcggtagtgaagatgaagcagacgggccaggtgtatgccatgaagatcatgaacaagtgggacatgctgaagaggggcgaggtgtcgtgcttccgtgaggagagggacgtgttggtgaatggggaccggcggtggatcacgcagctgcacttcgccttccaggatgagaactacctgtacctggtcatggagtattacgtgggcggggacctgctgacactgctgagcaagtttggggagcggattccggccgagatggcgcgcttctacctggcggagattgtcatggccatagactcggtgcaccggcttggctacgtgcacagggacatcaaacccgacaacatcctgctggaccgctgtggccacatccgcctggccgacttcggctcttgcctcaagctgcgggcagatggaacggtgcggtcgctggtggctgtgggcaccccagactacctgtcccccgagatcctgcaggctgtgggcggtgggcctgggacaggcagctacgggcccgagtgtgactggtgggcgctgggtgtattcgcctatgaaatgttctatgggcagacgcccttctacgcggattccacggcggagacctatggcaagatcgtccactacaaggagcacctctctctgccgctggtggacgaaggggtccctgaggaggctcgagacttcattcagcggttgctgtgtcccccggagacacggctgggccggggtggagcaggcgacttccggacacatcccttcttctttggcctcgactgggatggtctccgggacagcgtgcccccctttacaccggatttcgaaggtgccaccgacacatgcaacttcgacttggtggaggacgggctcactgccatggtgagcgggggcggggagacactgtcggacattcgggaaggtgcgccgctaggggtccacctgccttttgtgggctactcctactcctgcatggccctcagggacagtgaggtcccaggccccacacccatggaactggaggccgagcagctgcttgagccacacgtgcaagcgcccagcctggagccctcggtgtccccacaggatgaaacagctgaagtggcagttccagcggctgtccctgcggcagaggctgaggccgaggtgacgctgcgggagctccaggaagccctggaggaggaggtgctcacccggcagagcctgagccgggagatggaggccatccgcacggacaaccagaacttcgccagtcaactacgcgaggcagaggctcggaaccgggacctagaggcacacgtccggcagttgcaggagcggatggagttgctgcaggcagagggagccacagctgtcacgggggtccccagtccccgggccacggatccaccttcccatctagatggccccccggccgtggctgtgggccagtgcccgctggtggggccaggccccatgcaccgccgccacctgctgctccctgccagggtccctaggcctggcctatcggaggcgctttccctgctcctgttcgccgttgttctgtctcgtgccgccgccctgggctgcattgggttggtggcccacgccggccaactcaccgcagtctggcgccgcccaggagccgcccgcgctccctgaaccctagaactgtcttcgactccggggccccgttggaagactgagtgcccggggcacggcacagaagccgcgcccaccgcctgccagttcacaaccgctccgagcgtgggtctccgcccagctccagtcctgtgatccgggcccgccccctagcggccggggagggaggggccgggtccgcggccggcgaacggggctcgaagggtccttgtagccgggaatgctgctgctgctgctgctgctgctgctgctgctgctgctgctgctgctgctgctgctgctggggggatcacagaccatttctttctttcggccaggctgaggccctgacgtggatgggcaaactgcaggcctgggaaggcagcaagccgggccgtccgtgttccatcctccacgcacccccacctatcgttggttcgcaaagtgcaaagctttcttgtgcatgacgccctgctctggggagcgtctggcgcgatctctgcctgcttactcgggaaatttgcttttgccaaacccgctttttcggggatcccgcgcccccctcctcacttgcgctgctctcggagccccagccggctccgcccgcttcggcggtttggatatttattgacctcgtcctccgactcgctgacaggctacaggacccccaacaaccccaatccacgttttggatgcactgagaccccgacattcctcggtatttattgtctgtccccacctaggacccccacccccgaccctcgcgaataaaaggccctccatctgcccaaagctctgga